European Patent Specification EP 3 983 533 B1, published January 8, 2025. Title: Rational Therapeutic Targeting of Oncogenic Immune Signaling States in Myeloid Malignancies via the Ubiquitin Conjugating Enzyme UBE2N. Applicant: Starczynowski, Daniel Barreyro, Laura Seibel, William. The sequence listing filed with the application follows.

SEQUENCE LISTING (20 sequences)

SEQ ID NO: 1 - RNA, 22 nt, Artificial Sequence
  UBE2N forward primer sequence
tgatgtagcggagcagtggaag

SEQ ID NO: 2 - RNA, 22 nt, Artificial Sequence
  UBE2N reverse primer sequence
ggaggaagtcttggcagaacag

SEQ ID NO: 3 - RNA, 21 nt, Artificial Sequence
  FOS forward primer sequence
ccggggatagcctctcttact

SEQ ID NO: 4 - RNA, 19 nt, Artificial Sequence
  FOS reverse primer sequence
ccaggtccgtgcagaagtc

SEQ ID NO: 5 - RNA, 21 nt, Atificial Sequence
  JUN forward primer sequence
tccaagtgccgaaaaaggaag

SEQ ID NO: 6 - RNA, 21 nt, Artificial Sequence
  JUN reverse primer sequence
cgagttctgagctttcaaggt

SEQ ID NO: 7 - RNA, 21 nt, Artificial Sequence
  JUNB forward primer sequence
acaaactcctgaaaccgagcc

SEQ ID NO: 8 - RNA, 21 nt, Artificial Sequence
  JUNB reverse primer sequence
cgagccctgaccagaaaagta

SEQ ID NO: 9 - RNA, 21 nt, Artificial Sequence
  IL6 forward primer sequence
ggtacatcctcgacggcatct

SEQ ID NO: 10 - RNA, 21 nt, Artificial Sequence
  IL6 reverse primer sequence
gtgcctctttgctgctttcac

SEQ ID NO: 11 - RNA, 23 nt, Artificial Sequence
  IL1B forward primer sequence
aatctgtacctgtcctgcgtgtt

SEQ ID NO: 12 - RNA, 26 nt, Artificial Sequence
  IL1B reverse primer sequence
tgggtaatttttgggatctacactct

SEQ ID NO: 13 - RNA, 20 nt, Artificial Sequence
  TNF forward primer sequence
tcttctcgaaccccgagtga

SEQ ID NO: 14 - RNA, 19 nt, rArtificial Sequence
  TNF reverse primer sequence
cctctgatggcaccaccag

SEQ ID NO: 15 - RNA, 20 nt, Artificial Sequence
  Actin forward primer sequence
ctcttccagccttccttcct

SEQ ID NO: 16 - RNA, 20 nt, Artificial Sequence
  Actin reverse primer sequence
agcactgtgttggcgtacag

SEQ ID NO: 17 - RNA, 58 nt, Artificial Sequence
  UBE2N template oligonucleotide shUBE2N-2
ccggctaggctatatgccatgaatactcgagtattcatggcatatagcctagtttttg

SEQ ID NO: 18 - RNA, 58 nt, Artificial Sequence
  UBE2N template oligonucleotide shUBE2N-3
ccggagacaagttgggaagaatatgctcgagcatattcttcccaacttgtcttttttg

SEQ ID NO: 19 - RNA, 57 nt, Artificial Sequence
  UBE2N template oligonucleotide shUBE2N-1
ccgggctgaggcatttgtgagtcttctcgagaagactcacaaatgcctcagcttttt

SEQ ID NO: 20 - RNA, 57 nt, Artificial Sequence
  Non-silencing control shControl
ccggcaacaagatgaagagcaccaactcgagttggtgctcttcatcttgttgttttt